European Patent Specification EP 3 958 835 B1, published May 24, 2023. Title: Peptides for treatment of diabetes. Applicant: Follicum AB. The sequence listing filed with the application follows.

SEQUENCE LISTING (187 sequences)

SEQ ID NO: 1 - protein, 15 aa, Artificial Sequence
  Synthetic sequence
  MISC_FEATURE (1)..(15): peptide, FOL-005
VDTYDGDISVVYGLR

SEQ ID NO: 2 - protein, 15 aa, Artificial Sequence
  Synthetic sequence
  MISC_FEATURE (1)..(15): peptide
VDTYDGDISVVYGLS

SEQ ID NO: 3 - protein, 14 aa, Artificial Sequence
  Synthetic sequence
  MISC_FEATURE (1)..(14): peptide, FOL-025
VDTYDGDISVVYGL

SEQ ID NO: 4 - protein, 14 aa, Artificial Sequence
  Synthetic sequence
  MISC_FEATURE (1)..(14): peptide
DTYDGDISVVYGLR

SEQ ID NO: 5 - protein, 14 aa, Artificial Sequence
  Synthetic sequence
  MISC_FEATURE (1)..(14): peptide
TYDGDISVVYGLRS

SEQ ID NO: 6 - protein, 13 aa, Artificial Sequence
  Synthetic sequence
  MISC_FEATURE (1)..(13): peptide, FOL-024
VDTYDGDISVVYG

SEQ ID NO: 7 - protein, 13 aa, Artificial Sequence
  Synthetic sequence
  MISC_FEATURE (1)..(13): peptide
DTYDGDISVVYGL

SEQ ID NO: 8 - protein, 13 aa, Artificial Sequence
  Synthetic sequence
  MISC_FEATURE (1)..(13): peptide
TYDGDISVVYGLR

SEQ ID NO: 9 - protein, 13 aa, Artificial Sequence
  Synthetic sequence
  MISC_FEATURE (1)..(13): peptide
YDGDISVVYGLRS

SEQ ID NO: 10 - protein, 12 aa, Artificial Sequence
  Synthetic sequence
  MISC_FEATURE (1)..(12): peptide
VDTYDGDISVVY

SEQ ID NO: 11 - protein, 12 aa, Artificial Sequence
  Synthetic sequence
  MISC_FEATURE (1)..(12): peptide
DTYDGDISVVYG

SEQ ID NO: 12 - protein, 12 aa, Artificial Sequence
  Synthetic sequence
  MISC_FEATURE (1)..(12): peptide
TYDGDISVVYGL

SEQ ID NO: 13 - protein, 12 aa, Artificial Sequence
  Synthetic sequence
  MISC_FEATURE (1)..(12): peptide
YDGDISVVYGLR

SEQ ID NO: 14 - protein, 12 aa, Artificial Sequence
  Synthetic sequence
  MISC_FEATURE (1)..(12): peptide
DGDISVVYGLRS

SEQ ID NO: 15 - protein, 11 aa, Artificial Sequence
  Synthetic sequence
  MISC_FEATURE (1)..(11): peptide
VDTYDGDISVV

SEQ ID NO: 16 - protein, 11 aa, Artificial Sequence
  Synthetic sequence
  MISC_FEATURE (1)..(11): peptide
DTYDGDISVVY

SEQ ID NO: 17 - protein, 11 aa, Artificial Sequence
  Synthetic sequence
  MISC_FEATURE (1)..(11): peptide
TYDGDISVVYG

SEQ ID NO: 18 - protein, 11 aa, Artificial Sequence
  Synthetic sequence
  MISC_FEATURE (1)..(11): peptide
YDGDISVVYGL

SEQ ID NO: 19 - protein, 11 aa, Artificial Sequence
  Synthetic sequence
  MISC_FEATURE (1)..(11): peptide
DGDISVVYGLR

SEQ ID NO: 20 - protein, 11 aa, Artificial Sequence
  Synthetic sequence
  MISC_FEATURE (1)..(11): peptide
GDISVVYGLRS

SEQ ID NO: 21 - protein, 10 aa, Artificial Sequence
  Synthetic sequence
  MISC_FEATURE (1)..(10): peptide
VDTYDGDISV

SEQ ID NO: 22 - protein, 10 aa, Artificial Sequence
  Synthetic sequence
  MISC_FEATURE (1)..(10): peptide
DTYDGDISVV

SEQ ID NO: 23 - protein, 10 aa, Artificial Sequence
  Synthetic sequence
  MISC_FEATURE (1)..(10): peptide
TYDGDISVVY

SEQ ID NO: 24 - protein, 10 aa, Artificial Sequence
  Synthetic sequence
  MISC_FEATURE (1)..(10): peptide
YDGDISVVYG

SEQ ID NO: 25 - protein, 10 aa, Artificial Sequence
  Synthetic sequence
  MISC_FEATURE (1)..(10): peptide
DGDISVVYGL

SEQ ID NO: 26 - protein, 10 aa, Artificial Sequence
  Synthetic sequence
  MISC_FEATURE (1)..(10): peptide, FOL-009h
GDISVVYGLR

SEQ ID NO: 27 - protein, 10 aa, Artificial Sequence
  Synthetic sequence
  MISC_FEATURE (1)..(10): peptide
DISVVYGLRS

SEQ ID NO: 28 - protein, 9 aa, Artificial Sequence
  Synthetic sequence
  MISC_FEATURE (1)..(9): peptide, FOL-019h
VDTYDGDIS

SEQ ID NO: 29 - protein, 9 aa, Artificial Sequence
  Synthetic sequence
  MISC_FEATURE (1)..(9): peptide
DTYDGDISV

SEQ ID NO: 30 - protein, 9 aa, Artificial Sequence
  Synthetic sequence
  MISC_FEATURE (1)..(9): peptide
TYDGDISVV

SEQ ID NO: 31 - protein, 9 aa, Artificial Sequence
  Synthetic sequence
  MISC_FEATURE (1)..(9): peptide
YDGDISVVY

SEQ ID NO: 32 - protein, 9 aa, Artificial Sequence
  Synthetic sequence
  MISC_FEATURE (1)..(9): peptide
DGDISVVYG

SEQ ID NO: 33 - protein, 9 aa, Artificial Sequence
  Synthetic sequence
  MISC_FEATURE (1)..(9): peptide
GDISVVYGL

SEQ ID NO: 34 - protein, 9 aa, Artificial Sequence
  Synthetic sequence
  MISC_FEATURE (1)..(9): peptide
DISVVYGLR

SEQ ID NO: 35 - protein, 9 aa, Artificial Sequence
  Synthetic sequence
  MISC_FEATURE (1)..(9): peptide
ISVVYGLRS

SEQ ID NO: 36 - protein, 8 aa, Artificial Sequence
  Synthetic sequence
  MISC_FEATURE (1)..(8): peptide
VDTYDGDI

SEQ ID NO: 37 - protein, 8 aa, Artificial Sequence
  Synthetic sequence
  MISC_FEATURE (1)..(8): peptide
DTYDGDIS

SEQ ID NO: 38 - protein, 8 aa, Artificial Sequence
  Synthetic sequence
  MISC_FEATURE (1)..(8): peptide
TYDGDISV

SEQ ID NO: 39 - protein, 8 aa, Artificial Sequence
  Synthetic sequence
  MISC_FEATURE (1)..(8): peptide
YDGDISVV

SEQ ID NO: 40 - protein, 8 aa, Artificial Sequence
  Synthetic sequence
  MISC_FEATURE (1)..(8): peptide
DGDISVVY

SEQ ID NO: 41 - protein, 8 aa, Artificial Sequence
  Synthetic sequence
  MISC_FEATURE (1)..(8): peptide
GDISVVYG

SEQ ID NO: 42 - protein, 8 aa, Artificial Sequence
  Synthetic sequence
  MISC_FEATURE (1)..(8): peptide
DISVVYGL

SEQ ID NO: 43 - protein, 8 aa, Artificial Sequence
  Synthetic sequence
  MISC_FEATURE (1)..(8): peptide
ISVVYGLR

SEQ ID NO: 44 - protein, 7 aa, Artificial Sequence
  Synthetic sequence
  MISC_FEATURE (1)..(7): peptide
VDTYDGD

SEQ ID NO: 45 - protein, 7 aa, Artificial Sequence
  Synthetic sequence
  MISC_FEATURE (1)..(7): peptide
DTYDGDI

SEQ ID NO: 46 - protein, 7 aa, Artificial Sequence
  Synthetic sequence
  MISC_FEATURE (1)..(7): peptide
TYDGDIS

SEQ ID NO: 47 - protein, 7 aa, Artificial Sequence
  Synthetic sequence
  MISC_FEATURE (1)..(7): peptide
YDGDISV

SEQ ID NO: 48 - protein, 7 aa, Artificial Sequence
  Synthetic sequence
  MISC_FEATURE (1)..(7): peptide
DGDISVV

SEQ ID NO: 49 - protein, 7 aa, Artificial Sequence
  Synthetic sequence
  MISC_FEATURE (1)..(7): peptide
GDISVVY

SEQ ID NO: 50 - protein, 7 aa, Artificial Sequence
  Synthetic sequence
  MISC_FEATURE (1)..(7): peptide
DISVVYG

SEQ ID NO: 51 - protein, 7 aa, Artificial Sequence
  Synthetic sequence
  MISC_FEATURE (1)..(7): peptide
ISVVYGL

SEQ ID NO: 52 - protein, 6 aa, Artificial Sequence
  Synthetic sequence
  MISC_FEATURE (1)..(6): peptide
DTYDGD

SEQ ID NO: 53 - protein, 6 aa, Artificial Sequence
  Synthetic sequence
  MISC_FEATURE (1)..(6): peptide
TYDGDI

SEQ ID NO: 54 - protein, 6 aa, Artificial Sequence
  Synthetic sequence
  MISC_FEATURE (1)..(6): peptide
YDGDIS

SEQ ID NO: 55 - protein, 6 aa, Artificial Sequence
  Synthetic sequence
  MISC_FEATURE (1)..(6): peptide
DGDISV

SEQ ID NO: 56 - protein, 6 aa, Artificial Sequence
  Synthetic sequence
  MISC_FEATURE (1)..(6): peptide
GDISVV

SEQ ID NO: 57 - protein, 6 aa, Artificial Sequence
  Synthetic sequence
  MISC_FEATURE (1)..(6): peptide
DISVVY

SEQ ID NO: 58 - protein, 6 aa, Artificial Sequence
  Synthetic sequence
  MISC_FEATURE (1)..(6): peptide
ISVVYG

SEQ ID NO: 59 - protein, 5 aa, Artificial Sequence
  Synthetic sequence
  MISC_FEATURE (1)..(5): peptide
TYDGD

SEQ ID NO: 60 - protein, 5 aa, Artificial Sequence
  Synthetic sequence
  MISC_FEATURE (1)..(5): peptide
YDGDI

SEQ ID NO: 61 - protein, 5 aa, Artificial Sequence
  Synthetic sequence
  MISC_FEATURE (1)..(5): peptide
DGDIS

SEQ ID NO: 62 - protein, 5 aa, Artificial Sequence
  Synthetic sequence
  MISC_FEATURE (1)..(5): peptide
GDISV

SEQ ID NO: 63 - protein, 5 aa, Artificial Sequence
  Synthetic sequence
  MISC_FEATURE (1)..(5): peptide
DISVV

SEQ ID NO: 64 - protein, 5 aa, Artificial Sequence
  Synthetic sequence
  MISC_FEATURE (1)..(5): peptide
ISVVY

SEQ ID NO: 65 - protein, 5 aa, Artificial Sequence
  Synthetic sequence
  MISC_FEATURE (1)..(5): peptide
SVVYG

SEQ ID NO: 66 - protein, 300 aa, Homo sapiens
  MISC_FEATURE (1)..(300): Wildtype human osteopontin
MRIAVICFCLLGITCAIPVKQADSGSSEEKQLYNKYPDAVATWLNPDPSQKQNLLAPQTLPSKSNESHDHMDDMDDEDDDDHVDSQDSIDSNDSDDVDDTDDSHQSDESHHSDESDELVTDFPTDLPATEVFTPVVPTVDTYDGRGDSVVYGLRSKSKKFRRPDIQYPDATDEDITSHMESEELNGAYKAIPVAQDLNAPSDWDSRGKDSYETSQLDDQSAETHSHKQSRLYKRKANDESNEHSDVIDSQELSKVSREFHSHEFHSHEDMLVVDPKSKEEDKHLKFRISHELDSASSEVN

SEQ ID NO: 67 - protein, 16 aa, Artificial Sequence
  Synthetic sequence
  MISC_FEATURE (1)..(16): peptide, FOL-002
VDTYDGRGDSVVYGLR

SEQ ID NO: 68 - protein, 15 aa, Artificial Sequence
  Synthetic sequence
  MISC_FEATURE (1)..(15): peptide
  MISC_FEATURE (3)..(3): X is T or V
  MISC_FEATURE (4)..(4): X is Y or P
  MISC_FEATURE (5)..(5): X is D or N
  MISC_FEATURE (7)..(7): X is D or G
  MISC_FEATURE (8)..(8): X is I or G
  MISC_FEATURE (10)..(10): X is V or L
  MISC_FEATURE (11)..(11): X is V or A
VDXXXGXXSXXYGLR

SEQ ID NO: 69 - protein, 15 aa, Artificial Sequence
  Synthetic sequence
  MISC_FEATURE (1)..(15): peptide, FOL-004
VDVPNGDISLAYGLR

SEQ ID NO: 70 - protein, 15 aa, Artificial Sequence
  Synthetic sequence
  MISC_FEATURE (1)..(15): peptide
DVPNGDISLAYGLRS

SEQ ID NO: 71 - protein, 14 aa, Artificial Sequence
  Synthetic sequence
  MISC_FEATURE (1)..(14): peptide
VDVPNGDISLAYGL

SEQ ID NO: 72 - protein, 14 aa, Artificial Sequence
  Synthetic sequence
  MISC_FEATURE (1)..(14): peptide
DVPNGDISLAYGLR

SEQ ID NO: 73 - protein, 14 aa, Artificial Sequence
  Synthetic sequence
  MISC_FEATURE (1)..(14): peptide
VPNGDISLAYGLRS

SEQ ID NO: 74 - protein, 13 aa, Artificial Sequence
  Synthetic sequence
  MISC_FEATURE (1)..(13): peptide, FOL-017
VDVPNGDISLAYG

SEQ ID NO: 75 - protein, 13 aa, Artificial Sequence
  Synthetic sequence
  MISC_FEATURE (1)..(13): peptide
DVPNGDISLAYGL

SEQ ID NO: 76 - protein, 13 aa, Artificial Sequence
  Synthetic sequence
  MISC_FEATURE (1)..(13): peptide
VPNGDISLAYGLR

SEQ ID NO: 77 - protein, 13 aa, Artificial Sequence
  Synthetic sequence
  MISC_FEATURE (1)..(13): peptide
PNGDISLAYGLRS

SEQ ID NO: 78 - protein, 12 aa, Artificial Sequence
  Synthetic sequence
  MISC_FEATURE (1)..(12): peptide
VDVPNGDISLAY

SEQ ID NO: 79 - protein, 12 aa, Artificial Sequence
  Synthetic sequence
  MISC_FEATURE (1)..(12): peptide
DVPNGDISLAYG

SEQ ID NO: 80 - protein, 12 aa, Artificial Sequence
  Synthetic sequence
  MISC_FEATURE (1)..(12): peptide
VPNGDISLAYGL

SEQ ID NO: 81 - protein, 12 aa, Artificial Sequence
  Synthetic sequence
  MISC_FEATURE (1)..(12): peptide
PNGDISLAYGLR

SEQ ID NO: 82 - protein, 12 aa, Artificial Sequence
  Synthetic sequence
  MISC_FEATURE (1)..(12): peptide
NGDISLAYGLRS

SEQ ID NO: 83 - protein, 11 aa, Artificial Sequence
  Synthetic sequence
  MISC_FEATURE (1)..(11): peptide
VDVPNGDISLA

SEQ ID NO: 84 - protein, 11 aa, Artificial Sequence
  Synthetic sequence
  MISC_FEATURE (1)..(11): peptide
DVPNGDISLAY

SEQ ID NO: 85 - protein, 11 aa, Artificial Sequence
  Synthetic sequence
  MISC_FEATURE (1)..(11): peptide
VPNGDISLAYG

SEQ ID NO: 86 - protein, 11 aa, Artificial Sequence
  Synthetic sequence
  MISC_FEATURE (1)..(11): peptide
PNGDISLAYGL

SEQ ID NO: 87 - protein, 11 aa, Artificial Sequence
  Synthetic sequence
  MISC_FEATURE (1)..(11): peptide
NGDISLAYGLR

SEQ ID NO: 88 - protein, 11 aa, Artificial Sequence
  Synthetic sequence
  MISC_FEATURE (1)..(11): peptide
GDISLAYGLRS

SEQ ID NO: 89 - protein, 10 aa, Artificial Sequence
  Synthetic sequence
  MISC_FEATURE (1)..(10): peptide
VDVPNGDISL

SEQ ID NO: 90 - protein, 10 aa, Artificial Sequence
  Synthetic sequence
  MISC_FEATURE (1)..(10): peptide
DVPNGDISLA

SEQ ID NO: 91 - protein, 10 aa, Artificial Sequence
  Synthetic sequence
  MISC_FEATURE (1)..(10): peptide
VPNGDISLAY

SEQ ID NO: 92 - protein, 10 aa, Artificial Sequence
  Synthetic sequence
  MISC_FEATURE (1)..(10): peptide
PNGDISLAYG

SEQ ID NO: 93 - protein, 10 aa, Artificial Sequence
  Synthetic sequence
  MISC_FEATURE (1)..(10): peptide
NGDISLAYGL

SEQ ID NO: 94 - protein, 10 aa, Artificial Sequence
  Synthetic sequence
  MISC_FEATURE (1)..(10): peptide, FOL-009
GDISLAYGLR

SEQ ID NO: 95 - protein, 10 aa, Artificial Sequence
  Synthetic sequence
  MISC_FEATURE (1)..(10): peptide
DISLAYGLRS

SEQ ID NO: 96 - protein, 9 aa, Artificial Sequence
  Synthetic sequence
  MISC_FEATURE (1)..(9): peptide
  MISC_FEATURE (1)..(9): peptide, FOL-019
VDVPNGDIS

SEQ ID NO: 97 - protein, 9 aa, Artificial Sequence
  Synthetic sequence
  MISC_FEATURE (1)..(9): peptide
DVPNGDISL

SEQ ID NO: 98 - protein, 9 aa, Artificial Sequence
  Synthetic sequence
  MISC_FEATURE (1)..(9): peptide
VPNGDISLA

SEQ ID NO: 99 - protein, 9 aa, Artificial Sequence
  Synthetic sequence
  MISC_FEATURE (1)..(9): peptide
PNGDISLAY

SEQ ID NO: 100 - protein, 9 aa, Artificial Sequence
  Synthetic sequence
  MISC_FEATURE (1)..(9): peptide
NGDISLAYG

SEQ ID NO: 101 - protein, 9 aa, Artificial Sequence
  Synthetic sequence
  MISC_FEATURE (1)..(9): peptide
GDISLAYGL

SEQ ID NO: 102 - protein, 9 aa, Artificial Sequence
  Synthetic sequence
  MISC_FEATURE (1)..(9): peptide
DISLAYGLR

SEQ ID NO: 103 - protein, 9 aa, Artificial Sequence
  Synthetic sequence
  MISC_FEATURE (1)..(9): peptide
ISLAYGLRS

SEQ ID NO: 104 - protein, 8 aa, Artificial Sequence
  Synthetic sequence
  MISC_FEATURE (1)..(8): peptide
VDVPNGDI

SEQ ID NO: 105 - protein, 8 aa, Artificial Sequence
  Synthetic sequence
  MISC_FEATURE (1)..(8): peptide
DVPNGDIS

SEQ ID NO: 106 - protein, 8 aa, Artificial Sequence
  Synthetic sequence
  MISC_FEATURE (1)..(8): peptide
VPNGDISL

SEQ ID NO: 107 - protein, 8 aa, Artificial Sequence
  Synthetic sequence
  MISC_FEATURE (1)..(8): peptide
PNGDISLA

SEQ ID NO: 108 - protein, 8 aa, Artificial Sequence
  Synthetic sequence
  MISC_FEATURE (1)..(8): peptide
NGDISLAY

SEQ ID NO: 109 - protein, 8 aa, Artificial Sequence
  Synthetic sequence
  MISC_FEATURE (1)..(8): peptide
GDISLAYG

SEQ ID NO: 110 - protein, 8 aa, Artificial Sequence
  Synthetic sequence
  MISC_FEATURE (1)..(8): peptide
DISLAYGL

SEQ ID NO: 111 - protein, 8 aa, Artificial Sequence
  Synthetic sequence
  MISC_FEATURE (1)..(8): peptide
ISLAYGLR

SEQ ID NO: 112 - protein, 7 aa, Artificial Sequence
  Synthetic sequence
  MISC_FEATURE (1)..(7): peptide
VDVPNGD

SEQ ID NO: 113 - protein, 7 aa, Artificial Sequence
  Synthetic sequence
  MISC_FEATURE (1)..(7): peptide
DVPNGDI

SEQ ID NO: 114 - protein, 7 aa, Artificial Sequence
  Synthetic sequence
  MISC_FEATURE (1)..(7): peptide
VPNGDIS

SEQ ID NO: 115 - protein, 7 aa, Artificial Sequence
  Synthetic sequence
  MISC_FEATURE (1)..(7): peptide
PNGDISL

SEQ ID NO: 116 - protein, 7 aa, Artificial Sequence
  Synthetic sequence
  MISC_FEATURE (1)..(7): peptide
NGDISLA

SEQ ID NO: 117 - protein, 7 aa, Artificial Sequence
  Synthetic sequence
  MISC_FEATURE (1)..(7): peptide
GDISLAY

SEQ ID NO: 118 - protein, 7 aa, Artificial Sequence
  Synthetic sequence
  MISC_FEATURE (1)..(7): peptide
DISLAYG

SEQ ID NO: 119 - protein, 7 aa, Artificial Sequence
  Synthetic sequence
  MISC_FEATURE (1)..(7): peptide
ISLAYGL

SEQ ID NO: 120 - protein, 6 aa, Artificial Sequence
  Synthetic sequence
  MISC_FEATURE (1)..(6): peptide
DVPNGD

SEQ ID NO: 121 - protein, 6 aa, Artificial Sequence
  Synthetic sequence
  MISC_FEATURE (1)..(6): peptide
VPNGDI

SEQ ID NO: 122 - protein, 6 aa, Artificial Sequence
  Synthetic sequence
  MISC_FEATURE (1)..(6): peptide
PNGDIS

SEQ ID NO: 123 - protein, 6 aa, Artificial Sequence
  Synthetic sequence
  MISC_FEATURE (1)..(6): peptide
NGDISL

SEQ ID NO: 124 - protein, 6 aa, Artificial Sequence
  Synthetic sequence
  MISC_FEATURE (1)..(6): peptide
GDISLA

SEQ ID NO: 125 - protein, 6 aa, Artificial Sequence
  Synthetic sequence
  MISC_FEATURE (1)..(6): peptide
DISLAY

SEQ ID NO: 126 - protein, 6 aa, Artificial Sequence
  Synthetic sequence
  MISC_FEATURE (1)..(6): peptide
ISLAYG

SEQ ID NO: 127 - protein, 5 aa, Artificial Sequence
  Synthetic sequence
  MISC_FEATURE (1)..(5): peptide
VPNGD

SEQ ID NO: 128 - protein, 5 aa, Artificial Sequence
  Synthetic sequence
  MISC_FEATURE (1)..(5): peptide
PNGDI

SEQ ID NO: 129 - protein, 5 aa, Artificial Sequence
  Synthetic sequence
  MISC_FEATURE (1)..(5): peptide
NGDIS

SEQ ID NO: 130 - protein, 5 aa, Artificial Sequence
  Synthetic sequence
  MISC_FEATURE (1)..(5): peptide
GDISL

SEQ ID NO: 131 - protein, 5 aa, Artificial Sequence
  Synthetic sequence
  MISC_FEATURE (1)..(5): peptide
DISLA

SEQ ID NO: 132 - protein, 5 aa, Artificial Sequence
  Synthetic sequence
  MISC_FEATURE (1)..(5): peptide
ISLAY

SEQ ID NO: 133 - protein, 5 aa, Artificial Sequence
  Synthetic sequence
  MISC_FEATURE (1)..(5): peptide
SLAYG

SEQ ID NO: 134 - protein, 294 aa, Mus musculus
  MISC_FEATURE (1)..(294): Wildtype murine osteopontin
MRLAVICFCLFGIASSLPVKVTDSGSSEEKLYSLHPDPIATWLVPDPSQKQNLLAPQNAVSSEEKDDFKQETLPSNSNESHDHMDDDDDDDDDDGDHAESEDSVDSDESDESHHSDESDETVTASTQADTFTPIVPTVDVPNGRGDSLAYGLRSKSRSFQVSDEQYPDATDEDLTSHMKSGESKESLDVIPVAQLLSMPSDQDNNGKGSHESSQLDEPSLETHRLEHSKESQESADQSDVIDSQASSKASLEHQSHKFHSHKDKLVLDPKSKEDDRYLKFRISHELESSSSEVN

SEQ ID NO: 135 - protein, 16 aa, Artificial Sequence
  Synthetic sequence
  MISC_FEATURE (1)..(16): peptide, FOL-001
VDVPNGRGDSLAYGLR

SEQ ID NO: 136 - protein, 16 aa, Artificial Sequence
  Synthetic sequence
  MISC_FEATURE (1)..(16): peptide, FOL-014
KPLAEIDSIELSYGIK

SEQ ID NO: 137 - protein, 16 aa, Artificial Sequence
  Synthetic sequence
  MISC_FEATURE (1)..(16): peptide, FOL-003
GDPNDGRGDSVVYGLR

SEQ ID NO: 138 - protein, 15 aa, Artificial Sequence
  Synthetic sequence
  MISC_FEATURE (1)..(15): peptide, FOL-026
VDTYDGGISVVYGLR

SEQ ID NO: 139 - protein, 15 aa, Artificial Sequence
  Synthetic sequence
  MISC_FEATURE (1)..(15): peptide, FOL-027
VDTYDGDGSVVYGLR

SEQ ID NO: 140 - protein, 16 aa, Artificial Sequence
  Synthetic sequence
  MISC_FEATURE (1)..(16): peptide
  MISC_FEATURE (2)..(2): X is C, P or G
  MISC_FEATURE (5)..(5): X is E or G
  MISC_FEATURE (6)..(6): X is C, D or I
  MISC_FEATURE (7)..(7): X is D, I, S or G
  MISC_FEATURE (8)..(8): X is S, D or G
  MISC_FEATURE (10)..(10): X is E or G
  MISC_FEATURE (12)..(12): X is S or T
KXLAXXXXIXLXYGIK

SEQ ID NO: 141 - protein, 16 aa, Artificial Sequence
  Synthetic sequence
  MISC_FEATURE (1)..(16): peptide
KCLAECDSIELSYGIK

SEQ ID NO: 142 - protein, 8 aa, Artificial Sequence
  Synthetic sequence
  MISC_FEATURE (1)..(8): peptide
CLAEIDSC

SEQ ID NO: 143 - protein, 18 aa, Artificial Sequence
  Synthetic sequence
  MISC_FEATURE (1)..(18): peptide
CFKPLAEIDSIECSYGIK

SEQ ID NO: 144 - protein, 16 aa, Artificial Sequence
  Synthetic sequence
  MISC_FEATURE (1)..(16): peptide
KPLAEDISIELSYGIK

SEQ ID NO: 145 - protein, 16 aa, Artificial Sequence
  Synthetic sequence
  MISC_FEATURE (1)..(16): peptide
KPLAEISDIELSYGIK

SEQ ID NO: 146 - protein, 16 aa, Artificial Sequence
  Synthetic sequence
  MISC_FEATURE (1)..(16): peptide
KPLAEIGDIELSYGIK

SEQ ID NO: 147 - protein, 15 aa, Artificial Sequence
  Synthetic sequence
  MISC_FEATURE (1)..(15): peptide
KPLAEGDIELSYGIK

SEQ ID NO: 148 - protein, 13 aa, Artificial Sequence
  Synthetic sequence
  MISC_FEATURE (1)..(13): peptide
KPLAEIELSYGIK

SEQ ID NO: 149 - protein, 16 aa, Artificial Sequence
  Synthetic sequence
  MISC_FEATURE (1)..(16): peptide
KPLAEIDSIELTYGIK

SEQ ID NO: 150 - protein, 16 aa, Artificial Sequence
  Synthetic sequence
  MISC_FEATURE (1)..(16): peptide
KPLAEIDGIELSYGIK

SEQ ID NO: 151 - protein, 16 aa, Artificial Sequence
  Synthetic sequence
  MISC_FEATURE (1)..(16): peptide
KPLAEIDGIELTYGIK

SEQ ID NO: 152 - protein, 16 aa, Artificial Sequence
  Synthetic sequence
  MISC_FEATURE (1)..(16): peptide
KPLAEIGSIELSYGIK

SEQ ID NO: 153 - protein, 16 aa, Artificial Sequence
  Synthetic sequence
  MISC_FEATURE (1)..(16): peptide
KGLAEIDSIELSYGIK

SEQ ID NO: 154 - protein, 16 aa, Artificial Sequence
  Synthetic sequence
  MISC_FEATURE (1)..(16): peptide
KPLAGIDSIGLSYGIK

SEQ ID NO: 155 - protein, 16 aa, Artificial Sequence
  Synthetic sequence
  MISC_FEATURE (1)..(16): peptide
KCLAEIDSCELSYGIK

SEQ ID NO: 156 - protein, 13 aa, Artificial Sequence
  Synthetic sequence
  MISC_FEATURE (1)..(13): peptide
CFKPLAEIDSIEC

SEQ ID NO: 157 - protein, 15 aa, Artificial Sequence
  Synthetic sequence
  MISC_FEATURE (1)..(15): peptide
VDVPEGDISLAYGLR

SEQ ID NO: 158 - protein, 15 aa, Artificial Sequence
  Synthetic sequence
  MISC_FEATURE (1)..(15): peptide
LDGLVRAYDNISPVG

SEQ ID NO: 159 - protein, 14 aa, Artificial Sequence
  Synthetic sequence
  MISC_FEATURE (1)..(14): peptide
GDPNGDISVVYGLR

SEQ ID NO: 160 - protein, 15 aa, Artificial Sequence
  Synthetic sequence
  MISC_FEATURE (1)..(15): peptide
VDVPNGDISLAYRLR

SEQ ID NO: 161 - protein, 15 aa, Artificial Sequence
  Synthetic sequence
  MISC_FEATURE (1)..(15): peptide
VDVPEGDISLAYRLR

SEQ ID NO: 162 - protein, 16 aa, Artificial Sequence
  synthetic peptide
  MISC_FEATURE (1)..(16): peptide
  MISC_FEATURE (2)..(2): X is C, P or G
  MISC_FEATURE (5)..(5): X is E or G
  MISC_FEATURE (6)..(6): X is C, I or absent
  MISC_FEATURE (7)..(7): X is D, G or absent
  MISC_FEATURE (8)..(8): X is S, G or absent
  MISC_FEATURE (10)..(10): X is E or G
KXLAXXXXIXLSYGIK

SEQ ID NO: 163 - protein, 13 aa, Artificial Sequence
  synthetic peptide
  MISC_FEATURE (1)..(13): peptide
  MISC_FEATURE (2)..(2): X is C, P or G
  MISC_FEATURE (5)..(5): X is E or G
  MISC_FEATURE (7)..(7): X is E or G
KXLAXIXLSYGIK

SEQ ID NO: 164 - protein, 15 aa, Artificial Sequence
  synthetic peptide
  MISC_FEATURE (1)..(15): peptide
  MISC_FEATURE (5)..(5): X is E or N
  MISC_FEATURE (13)..(13): X is R or G
VDVPXGDISLAYXLR

SEQ ID NO: 165 - protein, 15 aa, Artificial Sequence
  synthetic peptide
  MISC_FEATURE (1)..(15): peptide
  MISC_FEATURE (7)..(7): X is D or G
  MISC_FEATURE (8)..(8): X is I or G
VDTYDGXXSVVYGLR

SEQ ID NO: 166 - protein, 16 aa, Artificial Sequence
  synthetic peptide
  MISC_FEATURE (1)..(16): peptide
  MISC_FEATURE (5)..(5): Z is D or G
  MISC_FEATURE (6)..(6): X is D or G
  MISC_FEATURE (7)..(7): X is I or R
  MISC_FEATURE (8)..(8): X is G or absent
  MISC_FEATURE (9)..(9): X is D or absent
GDPNXXXXXSVVYGLR

SEQ ID NO: 167 - protein, 15 aa, Artificial Sequence
  synthetic peptide
  MISC_FEATURE (1)..(15): peptide
  MISC_FEATURE (2)..(2): X is beta D
VXTYDGDISVVYGLR

SEQ ID NO: 168 - protein, 15 aa, Artificial Sequence
  synthetic peptide
  MISC_FEATURE (1)..(15): peptide
  MISC_FEATURE (5)..(5): X is beta D
VDTYXGDISVVYGLR

SEQ ID NO: 169 - protein, 15 aa, Artificial Sequence
  synthetic peptide
  MISC_FEATURE (1)..(15): peptide
  MISC_FEATURE (7)..(7): X is beta D
VDTYDGXISVVYGLR

SEQ ID NO: 170 - protein, 14 aa, Artificial Sequence
  synthetic sequence
  MISC_FEATURE (1)..(14): peptide
LAEIDSIELSYGIK

SEQ ID NO: 171 - protein, 13 aa, Artificial Sequence
  synthetic sequence
  MISC_FEATURE (1)..(13): peptide, FOL-056
AEIDSIELSYGIK

SEQ ID NO: 172 - protein, 12 aa, Artificial Sequence
  synthetic sequence
  MISC_FEATURE (1)..(12): peptide, FOL-057
EIDSIELSYGIK

SEQ ID NO: 173 - protein, 11 aa, Artificial Sequence
  synthetic sequence
  MISC_FEATURE (1)..(11): peptide, FOL-058
IDSIELSYGIK

SEQ ID NO: 174 - protein, 10 aa, Artificial Sequence
  synthetic sequence
  MISC_FEATURE (1)..(10): peptide, FOL-059
DSIELSYGIK

SEQ ID NO: 175 - protein, 9 aa, Artificial Sequence
  synthetic sequence
  MISC_FEATURE (1)..(9): peptide, FOL-060
SIELSYGIK

SEQ ID NO: 176 - protein, 8 aa, Artificial Sequence
  synthetic sequence
  MISC_FEATURE (1)..(8): peptide
IELSYGIK

SEQ ID NO: 177 - protein, 7 aa, Artificial Sequence
  synthetic sequence
  MISC_FEATURE (1)..(7): peptide
  MISC_FEATURE (1)..(1): X is E or G
  MISC_FEATURE (3)..(3): X is S or T
XLXYGIK

SEQ ID NO: 178 - protein, 9 aa, Artificial Sequence
  synthetic sequence
  MISC_FEATURE (1)..(9): peptide
  MISC_FEATURE (1)..(1): X is D or G
  MISC_FEATURE (2)..(2): X is I or G
  MISC_FEATURE (4)..(4): X is V or L
  MISC_FEATURE (5)..(5): X is V or A
XXSXXYGLR

SEQ ID NO: 179 - protein, 15 aa, Artificial Sequence
  synthetic sequence
  MISC_FEATURE (1)..(15): peptide
KPLAEIDSIELSYGI

SEQ ID NO: 180 - protein, 14 aa, Artificial Sequence
  synthetic sequence
  MISC_FEATURE (1)..(14): peptide
KPLAEIDSIELSYG

SEQ ID NO: 181 - protein, 13 aa, Artificial Sequence
  synthetic sequence
  MISC_FEATURE (1)..(13): peptide
KPLAEIDSIELSY

SEQ ID NO: 182 - protein, 12 aa, Artificial Sequence
  synthetic sequence
  MISC_FEATURE (1)..(12): peptide
KPLAEIDSIELS

SEQ ID NO: 183 - protein, 11 aa, Artificial Sequence
  synthetic sequence
  MISC_FEATURE (1)..(11): peptide
KPLAEIDSIEL

SEQ ID NO: 184 - protein, 10 aa, Artificial Sequence
  synthetic sequence
  MISC_FEATURE (1)..(10): peptide
KPLAEIDSIE

SEQ ID NO: 185 - protein, 25 aa, Artificial Sequence
  synthetic sequence
  MISC_FEATURE (1)..(25): peptide, FOL-199
GKYGFYTHVFRLKKWIQKVIDQFGE

SEQ ID NO: 186 - protein, 9 aa, Artificial Sequence
  synthetic sequence
  MISC_FEATURE (1)..(9): peptide, oxytocin
CYIQNCPLG

SEQ ID NO: 187 - protein, 37 aa, Artificial Sequence
  synthetic sequence
  MISC_FEATURE (1)..(37): peptide, LL-37
LLGDFFRKSKEKIGKEFKRIVQRIKDFLRNLVPRTES